European Patent Application EP 4 414 028 A2, published August 14, 2024. Title: Compositions for Treating Pathological Calcification Conditions, and Methods Using Same. Applicant: YALE UNIVERSITY. Application EM. The sequence listing filed with the application follows.

SEQUENCE LISTING (30 sequences)

SEQ ID NO: 1 - protein, 925 aa, Homo sapiens
MERDGCAGGGSRGGEGGRAPREGPAGNGRDRGRSHAAEAPGDPQAAASLLAPMDVGEEPLEKAARARTAKDPNTYKVLSLVLSVCVLTTILGCIFGLKPSCAKEVKSCKGRCFERTFGNCRCDAACVELGNCCLDYQETCIEPEHIWTCNKFRCGEKRLTRSLCACSDDCKDKGDCCINYSSVCQGEKSWVEEPCESINEPQCPAGFETPPTLLFSLDGFRAEYLHTWGGLLPVISKLKKCGTYTKNMRPVYPTKTFPNHYSIVTGLYPESHGIIDNKMYDPKMNASFSLKSKEKFNPEWYKGEPIWVTAKYQGLKSGTFFWPGSDVEINGIFPDIYKMYNGSVPFEERILAVLQWLQLPKDERPHFYTLYLEEPDSSGHSYGPVSSEVIKALQRVDGMVGMLMDGLKELNLHRCLNLILISDHGMEQGSCKKYIYLNKYLGDVKNIKVIYGPAARLRPSDVPDKYYSFNYEGIARNLSCREPNQHFKPYLKHFLPKRLHFAKSDRIEPLTFYLDPQWQLALNPSERKYCGSGFHGSDNVFSNMQALFVGYGPGFKHGIEADTFENIEVYNLMCDLLNLTPAPNNGTHGSLNHLLKNPVYTPKHPKEVHPLVQCPFTRNPRDNLGCSCNPSILPIEDFQTQFNLTVAEEKIIKHETLPYGRPRVLQKENTICLLSQHQFMSGYSQDILMPLWTSYTVDRNDSFSTEDFSNCLYQDFRIPLSPVHKCSFYKNNTKVSYGFLSPPQLNKNSSGIYSEALLTTNIVPMYQSFQVIWRYFHDTLLRKYAEERNGVNVVSGPVFDFDYDGRCDSLENLRQKRRVIRNQEILIPTHFFIVLTSCKDTSQTPLHCENLDTLAFILPHRTDNSESCVHGKHDSSWVEELLMLHRARITDVEHITGLSFYQQRKEPVSDILKLKTHLPTFSQED

SEQ ID NO: 2 - protein, 888 aa, Homo sapiens
MARRSSFQSCQIISLFTFAVGVNICLGFTAHRIKRAEGWEEGPPTVLSDSPWTNISGSCKGRCFELQEAGPPDCRCDNLCKSYTSCCHDFDELCLKTARGWECTKDRCGEVRNEENACHCSEDCLARGDCCTNYQVVCKGESHWVDDDCEEIKAAECPAGFVRPPLIIFSVDGFRASYMKKGSKVMPNIEKLRSCGTHSPYMRPVYPTKTFPNLYTLATGLYPESHGIVGNSMYDPVFDATFHLRGREKFNHRWWGGQPLWITATKQGVKAGTFFWSVVIPHERRILTILQWLTLPDHERPSVYAFYSEQPDFSGHKYGPFGPEMTNPLREIDKIVGQLMDGLKQLKLHRCVNVIFVGDHGMEDVTCDRTEFLSNYLTNVDDITLVPGTLGRIRSKFSNNAKYDPKAIIANLTCKKPDQHFKPYLKQHLPKRLHYANNRRIEDIHLLVERRWHVARKPLDVYKKPSGKCFFQGDHGFDNKVNSMQTVFVGYGSTFKYKTKVPPFENIELYNVMCDLLGLKPAPNNGTHGSLNHLLRTNTFRPTMPEEVTRPNYPGIMYLQSDFDLGCTCDDKVEPKNKLDELNKRLHTKGSTEAETRKFRGSRNENKENINGNFEPRKERHLLYGRPAVLYRTRYDILYHTDFESGYSEIFLMPLWTSYTVSKQAEVSSVPDHLTSCVRPDVRVSPSFSQNCLAYKNDKQMSYGFLFPPYLSSSPEAKYDAFLVTNMVPMYPAFKRVWNYFQRVLVKKYASERNGVNVISGPIFDYDYDGLHDTEDKIKQYVEGSSIPVPTHYYSIITSCLDFTQPADKCDGPLSVSSFILPHRPDNEESCNSSEDESKWVEELMKMHTARVRDIEHLTSLDFFRKTSRSYPEILTLKTYLHTYESEI

SEQ ID NO: 3 - protein, 453 aa, Homo sapiens
MKLLVILLFSGLITGFRSDSSSSLPPKLLLVSFDGFRADYLKNYEFPHLQNFIKEGVLVEHVKNVFITKTFPNHYSIVTGLYEESHGIVANSMYDAVTKKHFSDSNDKDPFWWNEAVPIWVTNQLQENRSSAAAMWPGTDVPIHDTISSYFMNYNSSVSFEERLNNITMWLNNSNPPVTFATLYWEEPDASGHKYGPEDKENMSRVLKKIDDLIGDLVQRLKMLGLWENLNVIITSDHGMTQCSQDRLINLDSCIDHSYYTLIDLSPVAAILPKINRTEVYNKLKNCSPHMNVYLKEDIPNRFYYQHNDRIQPIILVADEGWTIVLNESSQKLGDHGYDNSLPSMHPFLAAHGPAFHKGYKHSTINIVDIYPMMCHILGLKPHPNNGTFGHTKCLLVDQWCINLPEAIAIVIGSLLVLTMLTCLIIIMQNRLSVPRPFSRLQLQEDDDDPLIG

SEQ ID NO: 4-8 - skipped (5 entries)

SEQ ID NO: 9 - protein, 16 aa, synthetic construct
  REGION 1..16: note = chemically synthesized
DSSSEEKFLRRIGRFG

SEQ ID NO: 10 - protein, 12 aa, synthetic construct
  REGION 1..12: note = chemically synthesized
EEEEEEEPRGDT

SEQ ID NO: 11 - protein, 12 aa, synthetic construct
  REGION 1..12: note = chemically synthesized
APWHLSSQYSRT

SEQ ID NO: 12 - protein, 12 aa, synthetic construct
  REGION 1..12: note = chemically synthesized
STLPIPHEFSRE

SEQ ID NO: 13 - protein, 12 aa, synthetic construct
  REGION 1..12: note = chemically synthesized
VTKHLNQISQSY

SEQ ID NO: 14 - skipped

SEQ ID NO: 15 - protein, 925 aa, synthetic construct
  REGION 1..925: note = chemically synthesized
MERDGCAGGGSRGGEGGRAPREGPAGNGRDRGRSHAAEAPGDPQAAASLLAPMDVGEEPLEKAARARTAKDPNTYKIISLFTFAVGVNICLGFTAGLKPSCAKEVKSCKGRCFERTFGNCRCDAACVELGNCCLDYQETCIEPEHIWTCNKFRCGEKRLTRSLCACSDDCKDKGDCCINYSSVCQGEKSWVEEPCESINEPQCPAGFETPPTLLFSLDGFRAEYLHTWGGLLPVISKLKKCGTYTKNMRPVYPTKTFPNHYSIVTGLYPESHGIIDNKMYDPKMNASFSLKSKEKFNPEWYKGEPIWVTAKYQGLKSGTFFWPGSDVEINGIFPDIYKMYNGSVPFEERILAVLQWLQLPKDERPHFYTLYLEEPDSSGHSYGPVSSEVIKALQRVDGMVGMLMDGLKELNLHRCLNLILISDHGMEQGSCKKYIYLNKYLGDVKNIKVIYGPAARLRPSDVPDKYYSFNYEGIARNLSCREPNQHFKPYLKHFLPKRLHFAKSDRIEPLTFYLDPQWQLALNPSERKYCGSGFHGSDNVFSNMQALFVGYGPGFKHGIEADTFENIEVYNLMCDLLNLTPAPNNGTHGSLNHLLKNPVYTPKHPKEVHPLVQCPFTRNPRDNLGCSCNPSILPIEDFQTQFNLTVAEEKIIKHETLPYGRPRVLQKENTICLLSQHQFMSGYSQDILMPLWTSYTVDRNDSFSTEDFSNCLYQDFRIPLSPVHKCSFYKNNTKVSYGFLSPPQLNKNSSGIYSEALLTTNIVPMYQSFQVIWRYFHDTLLRKYAEERNGVNVVSGPVFDFDYDGRCDSLENLRQKRRVIRNQEILIPTHFFIVLTSCKDTSQTPLHCENLDTLAFILPHRTDNSESCVHGKHDSSWVEELLMLHRARITDVEHITGLSFYQQRKEPVSDILKLKTHLPTFSQED

SEQ ID NO: 16 - protein, 1155 aa, synthetic construct
  REGION 1..1155: note = chemically synthesized
MERDGCAGGGSRGGEGGRAPREGPAGNGRDRGRSHAAEAPGDPQAAASLLAPMDVGEEPLEKAARARTAKDPNTYKIISLFTFAVGVNICLGFTAGLKPSCAKEVKSCKGRCFERTFGNCRCDAACVELGNCCLDYQETCIEPEHIWTCNKFRCGEKRLTRSLCACSDDCKDKGDCCINYSSVCQGEKSWVEEPCESINEPQCPAGFETPPTLLFSLDGFRAEYLHTWGGLLPVISKLKKCGTYTKNMRPVYPTKTFPNHYSIVTGLYPESHGIIDNKMYDPKMNASFSLKSKEKFNPEWYKGEPIWVTAKYQGLKSGTFFWPGSDVEINGIFPDIYKMYNGSVPFEERILAVLQWLQLPKDERPHFYTLYLEEPDSSGHSYGPVSSEVIKALQRVDGMVGMLMDGLKELNLHRCLNLILISDHGMEQGSCKKYIYLNKYLGDVKNIKVIYGPAARLRPSDVPDKYYSFNYEGIARNLSCREPNQHFKPYLKHFLPKRLHFAKSDRIEPLTFYLDPQWQLALNPSERKYCGSGFHGSDNVFSNMQALFVGYGPGFKHGIEADTFENIEVYNLMCDLLNLTPAPNNGTHGSLNHLLKNPVYTPKHPKEVHPLVQCPFTRNPRDNLGCSCNPSILPIEDFQTQFNLTVAEEKIIKHETLPYGRPRVLQKENTICLLSQHQFMSGYSQDILMPLWTSYTVDRNDSFSTEDFSNCLYQDFRIPLSPVHKCSFYKNNTKVSYGFLSPPQLNKNSSGIYSEALLTTNIVPMYQSFQVIWRYFHDTLLRKYAEERNGVNVVSGPVFDFDYDGRCDSLENLRQKRRVIRNQEILIPTHFFIVLTSCKDTSQTPLHCENLDTLAFILPHRTDNSESCVHGKHDSSWVEELLMLHRARITDVEHITGLSFYQQRKEPVSDILKLKTHLPTFSQEDLINDKTHTCPPCPAPELLGGPSVFLFPPKPKDTLMISRTPEVTCVVVDVSHEDPEVKFNWYVDGVEVHNAKTKPREEQYNSTYRVVSVLTVLHQDWLNGKEYKCKVSNKALPAPIEKTISKAKGQPREPQVYTLPPSREEMTKNQVSLTCLVKGFYPSDIAVEWESNGQPENNYKTTPPVLDSDGSFFLYSKLTVDKSRWQQGNVFSCSVMHEALHNHYTQKSLSLSPGK

SEQ ID NO: 17 - protein, 852 aa, synthetic construct
  REGION 1..852: note = chemically synthesized
MRGPAVLLTVALATLLAPGAGAGLKPSCAKEVKSCKGRCFERTFGNCRCDAACVELGNCCLDYQETCIEPEHIWTCNKFRCGEKRLTRSLCACSDDCKDKGDCCINYSSVCQGEKSWVEEPCESINEPQCPAGFETPPTLLFSLDGFRAEYLHTWGGLLPVISKLKKCGTYTKNMRPVYPTKTFPNHYSIVTGLYPESHGIIDNKMYDPKMNASFSLKSKEKFNPEWYKGEPIWVTAKYQGLKSGTFFWPGSDVEINGIFPDIYKMYNGSVPFEERILAVLQWLQLPKDERPHFYTLYLEEPDSSGHSYGPVSSEVIKALQRVDGMVGMLMDGLKELNLHRCLNLILISDHGMEQGSCKKYIYLNKYLGDVKNIKVIYGPAARLRPSDVPDKYYSFNYEGIARNLSCREPNQHFKPYLKHFLPKRLHFAKSDRIEPLTFYLDPQWQLALNPSERKYCGSGFHGSDNVFSNMQALFVGYGPGFKHGIEADTFENIEVYNLMCDLLNLTPAPNNGTHGSLNHLLKNPVYTPKHPKEVHPLVQCPFTRNPRDNLGCSCNPSILPIEDFQTQFNLTVAEEKIIKHETLPYGRPRVLQKENTICLLSQHQFMSGYSQDILMPLWTSYTVDRNDSFSTEDFSNCLYQDFRIPLSPVHKCSFYKNNTKVSYGFLSPPQLNKNSSGIYSEALLTTNIVPMYQSFQVIWRYFHDTLLRKYAEERNGVNVVSGPVFDFDYDGRCDSLENLRQKRRVIRNQEILIPTHFFIVLTSCKDTSQTPLHCENLDTLAFILPHRTDNSESCVHGKHDSSWVEELLMLHRARITDVEHITGLSFYQQRKEPVSDILKLKTHLPTFSQED

SEQ ID NO: 18 - protein, 1082 aa, synthetic construct
  REGION 1..1082: note = chemically synthesized
MRGPAVLLTVALATLLAPGAGAGLKPSCAKEVKSCKGRCFERTFGNCRCDAACVELGNCCLDYQETCIEPEHIWTCNKFRCGEKRLTRSLCACSDDCKDKGDCCINYSSVCQGEKSWVEEPCESINEPQCPAGFETPPTLLFSLDGFRAEYLHTWGGLLPVISKLKKCGTYTKNMRPVYPTKTFPNHYSIVTGLYPESHGIIDNKMYDPKMNASFSLKSKEKFNPEWYKGEPIWVTAKYQGLKSGTFFWPGSDVEINGIFPDIYKMYNGSVPFEERILAVLQWLQLPKDERPHFYTLYLEEPDSSGHSYGPVSSEVIKALQRVDGMVGMLMDGLKELNLHRCLNLILISDHGMEQGSCKKYIYLNKYLGDVKNIKVIYGPAARLRPSDVPDKYYSFNYEGIARNLSCREPNQHFKPYLKHFLPKRLHFAKSDRIEPLTFYLDPQWQLALNPSERKYCGSGFHGSDNVFSNMQALFVGYGPGFKHGIEADTFENIEVYNLMCDLLNLTPAPNNGTHGSLNHLLKNPVYTPKHPKEVHPLVQCPFTRNPRDNLGCSCNPSILPIEDFQTQFNLTVAEEKIIKHETLPYGRPRVLQKENTICLLSQHQFMSGYSQDILMPLWTSYTVDRNDSFSTEDFSNCLYQDFRIPLSPVHKCSFYKNNTKVSYGFLSPPQLNKNSSGIYSEALLTTNIVPMYQSFQVIWRYFHDTLLRKYAEERNGVNVVSGPVFDFDYDGRCDSLENLRQKRRVIRNQEILIPTHFFIVLTSCKDTSQTPLHCENLDTLAFILPHRTDNSESCVHGKHDSSWVEELLMLHRARITDVEHITGLSFYQQRKEPVSDILKLKTHLPTFSQEDLINDKTHTCPPCPAPELLGGPSVFLFPPKPKDTLMISRTPEVTCVVVDVSHEDPEVKFNWYVDGVEVHNAKTKPREEQYNSTYRVVSVLTVLHQDWLNGKEYKCKVSNKALPAPIEKTISKAKGQPREPQVYTLPPSREEMTKNQVSLTCLVKGFYPSDIAVEWESNGQPENNYKTTPPVLDSDGSFFLYSKLTVDKSRWQQGNVFSCSVMHEALHNHYTQKSLSLSPGK

SEQ ID NO: 19 - protein, 849 aa, synthetic construct
  REGION 1..849: note = chemically synthesized
MRGPAVLLTVALATLLAPGAGAPSCAKEVKSCKGRCFERTFGNCRCDAACVELGNCCLDYQETCIEPEHIWTCNKFRCGEKRLTRSLCACSDDCKDKGDCCINYSSVCQGEKSWVEEPCESINEPQCPAGFETPPTLLFSLDGFRAEYLHTWGGLLPVISKLKKCGTYTKNMRPVYPTKTFPNHYSIVTGLYPESHGIIDNKMYDPKMNASFSLKSKEKFNPEWYKGEPIWVTAKYQGLKSGTFFWPGSDVEINGIFPDIYKMYNGSVPFEERILAVLQWLQLPKDERPHFYTLYLEEPDSSGHSYGPVSSEVIKALQRVDGMVGMLMDGLKELNLHRCLNLILISDHGMEQGSCKKYIYLNKYLGDVKNIKVIYGPAARLRPSDVPDKYYSFNYEGIARNLSCREPNQHFKPYLKHFLPKRLHFAKSDRIEPLTFYLDPQWQLALNPSERKYCGSGFHGSDNVFSNMQALFVGYGPGFKHGIEADTFENIEVYNLMCDLLNLTPAPNNGTHGSLNHLLKNPVYTPKHPKEVHPLVQCPFTRNPRDNLGCSCNPSILPIEDFQTQFNLTVAEEKIIKHETLPYGRPRVLQKENTICLLSQHQFMSGYSQDILMPLWTSYTVDRNDSFSTEDFSNCLYQDFRIPLSPVHKCSFYKNNTKVSYGFLSPPQLNKNSSGIYSEALLTTNIVPMYQSFQVIWRYFHDTLLRKYAEERNGVNVVSGPVFDFDYDGRCDSLENLRQKRRVIRNQEILIPTHFFIVLTSCKDTSQTPLHCENLDTLAFILPHRTDNSESCVHGKHDSSWVEELLMLHRARITDVEHITGLSFYQQRKEPVSDILKLKTHLPTFSQED

SEQ ID NO: 20 - protein, 1079 aa, synthetic construct
  REGION 1..1079: note = chemically synthesized
MRGPAVLLTVALATLLAPGAGAPSCAKEVKSCKGRCFERTFGNCRCDAACVELGNCCLDYQETCIEPEHIWTCNKFRCGEKRLTRSLCACSDDCKDKGDCCINYSSVCQGEKSWVEEPCESINEPQCPAGFETPPTLLFSLDGFRAEYLHTWGGLLPVISKLKKCGTYTKNMRPVYPTKTFPNHYSIVTGLYPESHGIIDNKMYDPKMNASFSLKSKEKFNPEWYKGEPIWVTAKYQGLKSGTFFWPGSDVEINGIFPDIYKMYNGSVPFEERILAVLQWLQLPKDERPHFYTLYLEEPDSSGHSYGPVSSEVIKALQRVDGMVGMLMDGLKELNLHRCLNLILISDHGMEQGSCKKYIYLNKYLGDVKNIKVIYGPAARLRPSDVPDKYYSFNYEGIARNLSCREPNQHFKPYLKHFLPKRLHFAKSDRIEPLTFYLDPQWQLALNPSERKYCGSGFHGSDNVFSNMQALFVGYGPGFKHGIEADTFENIEVYNLMCDLLNLTPAPNNGTHGSLNHLLKNPVYTPKHPKEVHPLVQCPFTRNPRDNLGCSCNPSILPIEDFQTQFNLTVAEEKIIKHETLPYGRPRVLQKENTICLLSQHQFMSGYSQDILMPLWTSYTVDRNDSFSTEDFSNCLYQDFRIPLSPVHKCSFYKNNTKVSYGFLSPPQLNKNSSGIYSEALLTTNIVPMYQSFQVIWRYFHDTLLRKYAEERNGVNVVSGPVFDFDYDGRCDSLENLRQKRRVIRNQEILIPTHFFIVLTSCKDTSQTPLHCENLDTLAFILPHRTDNSESCVHGKHDSSWVEELLMLHRARITDVEHITGLSFYQQRKEPVSDILKLKTHLPTFSQEDLINDKTHTCPPCPAPELLGGPSVFLFPPKPKDTLMISRTPEVTCVVVDVSHEDPEVKFNWYVDGVEVHNAKTKPREEQYNSTYRVVSVLTVLHQDWLNGKEYKCKVSNKALPAPIEKTISKAKGQPREPQVYTLPPSREEMTKNQVSLTCLVKGFYPSDIAVEWESNGQPENNYKTTPPVLDSDGSFFLYSKLTVDKSRWQQGNVFSCSVMHEALHNHYTQKSLSLSPGK

SEQ ID NO: 21 - protein, 1550 aa, synthetic construct
  REGION 1..1550: note = chemically synthesized
MERDGCAGGGSRGGEGGRAPREGPAGNGRDRGRSHAAEAPGDPQAAASLLAPMDVGEEPLEKAARARTAKDPNTYKIISLFTFAVGVNICLGFTAGLKPSCAKEVKSCKGRCFERTFGNCRCDAACVELGNCCLDYQETCIEPEHIWTCNKFRCGEKRLTRSLCACSDDCKDKGDCCINYSSVCQGEKSWVEEPCESINEPQCPAGFETPPTLLFSLDGFRAEYLHTWGGLLPVISKLKKCGTYTKNMRPVYPTKTFPNHYSIVTGLYPESHGIIDNKMYDPKMNASFSLKSKEKFNPEWYKGEPIWVTAKYQGLKSGTFFWPGSDVEINGIFPDIYKMYNGSVPFEERILAVLQWLQLPKDERPHFYTLYLEEPDSSGHSYGPVSSEVIKALQRVDGMVGMLMDGLKELNLHRCLNLILISDHGMEQGSCKKYIYLNKYLGDVKNIKVIYGPAARLRPSDVPDKYYSFNYEGIARNLSCREPNQHFKPYLKHFLPKRLHFAKSDRIEPLTFYLDPQWQLALNPSERKYCGSGFHGSDNVFSNMQALFVGYGPGFKHGIEADTFENIEVYNLMCDLLNLTPAPNNGTHGSLNHLLKNPVYTPKHPKEVHPLVQCPFTRNPRDNLGCSCNPSILPIEDFQTQFNLTVAEEKIIKHETLPYGRPRVLQKENTICLLSQHQFMSGYSQDILMPLWTSYTVDRNDSFSTEDFSNCLYQDFRIPLSPVHKCSFYKNNTKVSYGFLSPPQLNKNSSGIYSEALLTTNIVPMYQSFQVIWRYFHDTLLRKYAEERNGVNVVSGPVFDFDYDGRCDSLENLRQKRRVIRNQEILIPTHFFIVLTSCKDTSQTPLHCENLDTLAFILPHRTDNSESCVHGKHDSSWVEELLMLHRARITDVEHITGLSFYQQRKEPVSDILKLKTHLPTFSQEDRSGSGGSMKWVTFLLLLFVSGSAFSRGVFRREAHKSEIAHRYNDLGEQHFKGLVLIAFSQYLQKCSYDEHAKLVQEVTDFAKTCVADESAANCDKSLHTLFGDKLCAIPNLRENYGELADCCTKQEPERNECFLQHKDDNPSLPPFERPEAEAMCTSFKENPTTFMGHYLHEVARRHPYFYAPELLYYAEQYNEILTQCCAEADKESCLTPKLDGVKEKALVSSVRQRMKCSSMQKFGERAFKAWAVARLSQTFPNADFAEITKLATDLTKVNKECCHGDLLECADDRAELAKYMCENQATISSKLQTCCDKPLLKKAHCLSEVEHDTMPADLPAIAADFVEDQEVCKNYAEAKDVFLGTFLYEYSRRHPDYSVSLLLRLAKKYEATLEKCCAEANPPACYGTVLAEFQPLVEEPKNLVKTNCDLYEKLGEYGFQNAILVRYTQKAPQVSTPTLVEAARNLGRVGTKCCTLPEDQRLPCVEDYLSAILNRVCLLHEKTPVSEHVTKCCSGSLVERRPCFSALTVDETYVPKEFKAETFTFHSDICTLPEKEKQIKKQTALAELVKHKPKATAEQLKTVMDDFAQFLDTCCKAADKDTCFSTEGPNLVTRCKDALARSWSHPQFEK

SEQ ID NO: 22 - protein, 1474 aa, synthetic construct
  REGION 1..1474: note = chemically synthesized
MRGPAVLLTVALATLLAPGAGAPSCAKEVKSCKGRCFERTFGNCRCDAACVELGNCCLDYQETCIEPEHIWTCNKFRCGEKRLTRSLCACSDDCKDKGDCCINYSSVCQGEKSWVEEPCESINEPQCPAGFETPPTLLFSLDGFRAEYLHTWGGLLPVISKLKKCGTYTKNMRPVYPTKTFPNHYSIVTGLYPESHGIIDNKMYDPKMNASFSLKSKEKFNPEWYKGEPIWVTAKYQGLKSGTFFWPGSDVEINGIFPDIYKMYNGSVPFEERILAVLQWLQLPKDERPHFYTLYLEEPDSSGHSYGPVSSEVIKALQRVDGMVGMLMDGLKELNLHRCLNLILISDHGMEQGSCKKYIYLNKYLGDVKNIKVIYGPAARLRPSDVPDKYYSFNYEGIARNLSCREPNQHFKPYLKHFLPKRLHFAKSDRIEPLTFYLDPQWQLALNPSERKYCGSGFHGSDNVFSNMQALFVGYGPGFKHGIEADTFENIEVYNLMCDLLNLTPAPNNGTHGSLNHLLKNPVYTPKHPKEVHPLVQCPFTRNPRDNLGCSCNPSILPIEDFQTQFNLTVAEEKIIKHETLPYGRPRVLQKENTICLLSQHQFMSGYSQDILMPLWTSYTVDRNDSFSTEDFSNCLYQDFRIPLSPVHKCSFYKNNTKVSYGFLSPPQLNKNSSGIYSEALLTTNIVPMYQSFQVIWRYFHDTLLRKYAEERNGVNVVSGPVFDFDYDGRCDSLENLRQKRRVIRNQEILIPTHFFIVLTSCKDTSQTPLHCENLDTLAFILPHRTDNSESCVHGKHDSSWVEELLMLHRARITDVEHITGLSFYQQRKEPVSDILKLKTHLPTFSQEDRSGSGGSMKWVTFLLLLFVSGSAFSRGVFRREAHKSEIAHRYNDLGEQHFKGLVLIAFSQYLQKCSYDEHAKLVQEVTDFAKTCVADESAANCDKSLHTLFGDKLCAIPNLRENYGELADCCTKQEPERNECFLQHKDDNPSLPPFERPEAEAMCTSFKENPTTFMGHYLHEVARRHPYFYAPELLYYAEQYNEILTQCCAEADKESCLTPKLDGVKEKALVSSVRQRMKCSSMQKFGERAFKAWAVARLSQTFPNADFAEITKLATDLTKVNKECCHGDLLECADDRAELAKYMCENQATISSKLQTCCDKPLLKKAHCLSEVEHDTMPADLPAIAADFVEDQEVCKNYAEAKDVFLGTFLYEYSRRHPDYSVSLLLRLAKKYEATLEKCCAEANPPACYGTVLAEFQPLVEEPKNLVKTNCDLYEKLGEYGFQNAILVRYTQKAPQVSTPTLVEAARNLGRVGTKCCTLPEDQRLPCVEDYLSAILNRVCLLHEKTPVSEHVTKCCSGSLVERRPCFSALTVDETYVPKEFKAETFTFHSDICTLPEKEKQIKKQTALAELVKHKPKATAEQLKTVMDDFAQFLDTCCKAADKDTCFSTEGPNLVTRCKDALARSWSHPQFEK

SEQ ID NO: 23 - protein, 19 aa, synthetic construct
  REGION 1..19: note = chemically synthesized
IISLFTFAVGVNICLGFTA

SEQ ID NO: 24 - protein, 850 aa, synthetic construct
  REGION 1..850: note = chemically synthesized
MTSKFLLVSFILAALSLSTTFSLQPSCAKEVKSCKGRCFERTFSNCRCDAACVSLGNCCLDFQETCVEPTHIWTCNKFRCGEKRLSRFVCSCADDCKTHNDCCINYSSVCQDKKSWVEETCESIDTPECPAEFESPPTLLFSLDGFRAEYLHTWGGLLPVISKLKNCGTYTKNMRPMYPTKTFPNHYSIVTGLYPESHGIIDNKMYDPKMNASFSLKSKEKFNPLWYKGQPIWVTANHQEVKSGTYFWPGSDVEIDGILPDIYKVYNGSVPFEERILAVLEWLQLPSHERPHFYTLYLEEPDSSGHSHGPVSSEVIKALQKVDRLVGMLMDGLKDLGLDKCLNLILISDHGMEQGSCKKYVYLNKYLGDVNNVKVVYGPAARLRPTDVPETYYSFNYEALAKNLSCREPNQHFRPYLKPFLPKRLHFAKSDRIEPLTFYLDPQWQLALNPSERKYCGSGFHGSDNLFSNMQALFIGYGPAFKHGAEVDSFENIEVYNLMCDLLGLIPAPNNGSHGSLNHLLKKPIYNPSHPKEEGFLSQCPIKSTSNDLGCTCDPWIVPIKDFEKQLNLTTEDVDDIYHMTVPYGRPRILLKQHRVCLLQQQQFLTGYSLDLLMPLWASYTFLSNDQFSRDDFSNCLYQDLRIPLSPVHKCSYYKSNSKLSYGFLTPPRLNRVSNHIYSEALLTSNIVPMYQSFQVIWHYLHDTLLQRYAHERNGINVVSGPVFDFDYDGRYDSLEILKQNSRVIRSQEILIPTHFFIVLTSCKQLSETPLECSALESSAYILPHRPDNIESCTHGKRESSWVEELLTLHRARVTDVELITGLSFYQDRQESVSELLRLKTHLPIFSQED

SEQ ID NO: 25 - protein, 1474 aa, synthetic construct
  REGION 1..1474: note = chemically synthesized
MTSKFLLVSFILAALSLSTTFSLQPSCAKEVKSCKGRCFERTFSNCRCDAACVSLGNCCLDFQETCVEPTHIWTCNKFRCGEKRLSRFVCSCADDCKTHNDCCINYSSVCQDKKSWVEETCESIDTPECPAEFESPPTLLFSLDGFRAEYLHTWGGLLPVISKLKNCGTYTKNMRPMYPTKTFPNHYSIVTGLYPESHGIIDNKMYDPKMNASFSLKSKEKFNPLWYKGQPIWVTANHQEVKSGTYFWPGSDVEIDGILPDIYKVYNGSVPFEERILAVLEWLQLPSHERPHFYTLYLEEPDSSGHSHGPVSSEVIKALQKVDRLVGMLMDGLKDLGLDKCLNLILISDHGMEQGSCKKYVYLNKYLGDVNNVKVVYGPAARLRPTDVPETYYSFNYEALAKNLSCREPNQHFRPYLKPFLPKRLHFAKSDRIEPLTFYLDPQWQLALNPSERKYCGSGFHGSDNLFSNMQALFIGYGPAFKHGAEVDSFENIEVYNLMCDLLGLIPAPNNGSHGSLNHLLKKPIYNPSHPKEEGFLSQCPIKSTSNDLGCTCDPWIVPIKDFEKQLNLTTEDVDDIYHMTVPYGRPRILLKQHRVCLLQQQQFLTGYSLDLLMPLWASYTFLSNDQFSRDDFSNCLYQDLRIPLSPVHKCSYYKSNSKLSYGFLTPPRLNRVSNHIYSEALLTSNIVPMYQSFQVIWHYLHDTLLQRYAHERNGINVVSGPVFDFDYDGRYDSLEILKQNSRVIRSQEILIPTHFFIVLTSCKQLSETPLECSALESSAYILPHRPDNIESCTHGKRESSWVEELLTLHRARVTDVELITGLSFYQDRQESVSELLRLKTHLPIFSQEDGGSGGSMKWVTFLLLLFVSGSAFSRGVFRREAHKSEIAHRYNDLGEQHFKGLVLIAFSQYLQKCSYDEHAKLVQEVTDFAKTCVADESAANCDKSLHTLFGDKLCAIPNLRENYGELADCCTKQEPERNECFLQHKDDNPSLPPFERPEAEAMCTSFKENPTTFMGHYLHEVARRHPYFYAPELLYYAEQYNEILTQCCAEADKESCLTPKLDGVKEKALVSSVRQRMKCSSMQKFGERAFKAWAVARLSQTFPNADFAEITKLATDLTKVNKECCHGDLLECADDRAELAKYMCENQATISSKLQTCCDKPLLKKAHCLSEVEHDTMPADLPAIAADFVEDQEVCKNYAEAKDVFLGTFLYEYSRRHPDYSVSLLLRLAKKYEATLEKCCAEANPPACYGTVLAEFQPLVEEPKNLVKTNCDLYEKLGEYGFQNAILVRYTQKAPQVSTPTLVEAARNLGRVGTKCCTLPEDQRLPCVEDYLSAILNRVCLLHEKTPVSEHVTKCCSGSLVERRPCFSALTVDETYVPKEFKAETFTFHSDICTLPEKEKQIKKQTALAELVKHKPKATAEQLKTVMDDFAQFLDTCCKAADKDTCFSTEGPNLVTRCKDALARSWSHPQFEK

SEQ ID NO: 26 - protein, 227 aa, synthetic construct
  REGION 1..227: note = chemically synthesized
DKTHTCPPCPAPELLGGPSVFLFPPKPKDTLMISRTPEVTCVVVDVSHEDPEVKFNWYVDGVEVHNAKTKPREEQYNSTYRVVSVLTVLHQDWLNGKEYKCKVSNKALPAPIEKTISKAKGQPREPQVYTLPPSREEMTKNQVSLTCLVKGFYPSDIAVEWESNGQPENNYKTTPPVLDSDGSFFLYSKLTVDKSRWQQGNVFSCSVMHEALHNHYTQKSLSLSPGK

SEQ ID NO: 27 - protein, 618 aa, synthetic construct
  REGION 1..618: note = chemically synthesized
MKWVTFLLLLFVSGSAFSRGVFRREAHKSEIAHRYNDLGEQHFKGLVLIAFSQYLQKCSYDEHAKLVQEVTDFAKTCVADESAANCDKSLHTLFGDKLCAIPNLRENYGELADCCTKQEPERNECFLQHKDDNPSLPPFERPEAEAMCTSFKENPTTFMGHYLHEVARRHPYFYAPELLYYAEQYNEILTQCCAEADKESCLTPKLDGVKEKALVSSVRQRMKCSSMQKFGERAFKAWAVARLSQTFPNADFAEITKLATDLTKVNKECCHGDLLECADDRAELAKYMCENQATISSKLQTCCDKPLLKKAHCLSEVEHDTMPADLPAIAADFVEDQEVCKNYAEAKDVFLGTFLYEYSRRHPDYSVSLLLRLAKKYEATLEKCCAEANPPACYGTVLAEFQPLVEEPKNLVKTNCDLYEKLGEYGFQNAILVRYTQKAPQVSTPTLVEAARNLGRVGTKCCTLPEDQRLPCVEDYLSAILNRVCLLHEKTPVSEHVTKCCSGSLVERRPCFSALTVDETYVPKEFKAETFTFHSDICTLPEKEKQIKKQTALAELVKHKPKATAEQLKTVMDDFAQFLDTCCKAADKDTCFSTEGPNLVTRCKDALARSWSHPQFEK

SEQ ID NO: 28 - skipped

SEQ ID NO: 29 - protein, 6 aa, synthetic construct
  REGION 1..6: note = chemically synthesized
GGSGGS

SEQ ID NO: 30 - protein, 7 aa, synthetic construct
  REGION 1..7: note = chemically synthesized
RSGSGGS